European Patent Application EP 4 212 167 A1, published July 19, 2023. Title: Peptide composition for preventing or treating Alzheimer's disease. Applicant: DanDi Bioscience Inc. The sequence listing filed with the application follows.

SEQUENCE LISTING (10 sequences)

SEQ ID NO: 1 - protein, 11 aa, Artificial Sequence
  DD-S052
  BINDING (11): amine group (NH2) is added to C-terminus of polypeptide.
  SITE (9): trifluoroacetic acid (TFA) at a terminus of the 9th amino acid from the N terminus of a peptide is substituted with an acetate salt.
KLRVKLRRYLR

SEQ ID NO: 2 - protein, 11 aa, Artificial Sequence
  DD-S052P
  BINDING (11): amine group (NH2) is added to C-terminus of polypeptide.
  SITE (9): trifluoroacetic acid (TFA) at a terminus of the 9th amino acid from the N terminus of a peptide is substituted with an acetate salt.
  SITE (1): peptide N-terminus PEGylation
KLRVKLRRYLR

SEQ ID NO: 3 - protein, 11 aa, Artificial Sequence
  FP1 (WT)
KLGVEAKRYLD

SEQ ID NO: 4 - protein, 11 aa, Artificial Sequence
  FP3
KLGVEAKRYLR

SEQ ID NO: 5 - protein, 11 aa, Artificial Sequence
  FP13-NH2
  BINDING (11): amine group (NH2) is added to C-terminus of polypeptide.
KLRVKLRRYLR

SEQ ID NO: 6 - DNA, 21 bp, Artificial Sequence
  IL-1beta forward primer
ccttccaggatgaggacatga

SEQ ID NO: 7 - DNA, 21 bp, Artificial Sequence
  IL-1beta reverse primer
tgagtcacagaggatgggctc

SEQ ID NO: 8 - DNA, 20 bp, Artificial Sequence
  TNF-alpha forward primer
tcgtagcaaaccaccaagtg

SEQ ID NO: 9 - DNA, 20 bp, Artificial Sequence
  TNF-alpha reverse primer
atatagcaaatcggctgacg

SEQ ID NO: 10 - protein, 12 aa, Artificial Sequence
  polypeptide of claim 1 or 9
  VARIANT (1): /replace=""
  VARIANT (2): /replace="Arg"
  VARIANT (4): /replace="Arg"
  VARIANT (6): /replace="Lys"
  VARIANT (7): /replace="Leu"
  VARIANT (8): /replace="Arg"/replace="Leu"
  VARIANT (10): /replace="Ala"/replace="Trp"/replace="Lys"/replace="Asp"
  VARIANT (12): /replace="Arg"
LKLGVEAKRYLD